European Patent Specification EP 2 707 021 B1, published February 21, 2024. Title: GENETICALLY ENGINEERED GROWTH FACTOR VARIANTS. Applicant: MINERVA BIOTECHNOLOGIES CORP. Bamdad, Cynthia. The sequence listing filed with the application follows.

SEQUENCE LISTING (158 sequences)

SEQ ID NO: 1 - protein, 45 aa, Artificial Sequence
  Extra cellular domain of MUC1*
GTINVHDVETQFNQYKTEAASRYNLTISDVSVSDVPFPFSAQSGA

SEQ ID NO: 2 - protein, 45 aa, Artificial Sequence
  Extra cellular domain of MUC1*
GTINVHDVETQFNQYKTEAASPYNLTISDVSVSDVPFPFSAQSGA

SEQ ID NO: 3 - DNA, 32 bp, Artificial Sequence
  Primer for NM23
atcgatcatatggccaactgtgagcgtacctt

SEQ ID NO: 4 - DNA, 31 bp, Artificial Sequence
  Primer for NM23
gtggtgctcgagttcatagatccagttctga

SEQ ID NO: 5 - DNA, 30 bp, Artificial Sequence
  Primer for NM23
gcaggaacattatacatggcggtgattctg

SEQ ID NO: 6 - DNA, 30 bp, Artificial Sequence
  Primer for NM23
gccatgtataatgttcctgccaacttgtat

SEQ ID NO: 7 - DNA, 29 bp, Artificial Sequence
  Primer for NM23-H1 mutant P96S (proline #96 mutated to a serine)
tcggggagaccaactctgcagactccaag

SEQ ID NO: 8 - DNA, 29 bp, Artificial Sequence
  Primer for NM23-H1 mutant P96S (proline #96 mutated to a serine)
cttggagtctgcagagttggtctccccga

SEQ ID NO: 9 - DNA, 33 bp, Artificial Sequence
  Primer for NM23 P96S  C1
atcgatcatatggccaactgtgagcgtaccttc

SEQ ID NO: 10 - DNA, 33 bp, Artificial Sequence
  Primer for NM23 P96S  C1
gtggtgaccggtatagatccagttctgagcaca

SEQ ID NO: 11 - DNA, 33 bp, Artificial Sequence; identical to SEQ ID NO: 9
  Primer for NM23 P96S  C2

SEQ ID NO: 12 - DNA, 33 bp, Artificial Sequence
  Primer for NM23 P96S  C2
gtggtgaccggtgatccagttctgagcacagct

SEQ ID NO: 13 - DNA, 33 bp, Artificial Sequence; identical to SEQ ID NO: 9
  Primer for NM23 P96S  C6

SEQ ID NO: 14 - DNA, 35 bp, Artificial Sequence
  Primer for NM23 P96S  C6
gtggtgaccggtagcacagctcgtgtaatctacca

SEQ ID NO: 15 - DNA, 32 bp, Artificial Sequence; identical to SEQ ID NO: 3
  Primer for NM23 S120G GS2 linker

SEQ ID NO: 16 - DNA, 71 bp, Artificial Sequence
  Primer for NM23 S120G GS2 linker
atcgatgctagcggatccgccaccgccggatccgccaccgccttcatagatccagttctgagcacagctcg

SEQ ID NO: 17 - DNA, 36 bp, Artificial Sequence
  Primer for NM23 S120G fragment
atcgatgctagcatggccaactgtgagcgtaccttc

SEQ ID NO: 18 - DNA, 31 bp, Artificial Sequence; identical to SEQ ID NO: 4
  Primer for NM23 S120G

SEQ ID NO: 19 - DNA, 32 bp, Artificial Sequence; identical to SEQ ID NO: 3
  Primer for NM23 S120G GS3 linker

SEQ ID NO: 20 - DNA, 85 bp, Artificial Sequence
  Primer for NM23 S120G GS3 linker
atcgatgctagcggatccgccaccgccggatccgccaccgccggatccgccaccgcttcatagatccagttctgagcacagctcg

SEQ ID NO: 21 - DNA, 36 bp, Artificial Sequence; identical to SEQ ID NO: 17
  Primer for NM23 S120G

SEQ ID NO: 22 - DNA, 31 bp, Artificial Sequence; identical to SEQ ID NO: 4
  Primer for NM23 S120G

SEQ ID NO: 23 - DNA, 32 bp, Artificial Sequence; identical to SEQ ID NO: 3
  Primer for NM23 S120G IgG1h noC (modified hinge region of IgG1 without cysteines)

SEQ ID NO: 24 - DNA, 67 bp, Artificial Sequence
  Primer for NM23 S120G IgG1h noC (modified hinge region of IgG1 without cysteines)
tccggcgccggttttggcggtttagtatgggttttatcttcatagatccagttctgagcacagctcg

SEQ ID NO: 25 - DNA, 32 bp, Artificial Sequence; identical to SEQ ID NO: 3
  Primer for NM23 S120G IgG1h noC (modified hinge region of IgG1 without cysteines)

SEQ ID NO: 26 - DNA, 65 bp, Artificial Sequence
  Primer for NM23 S120G IgG1h noC (modified hinge region of IgG1 without cysteines)
atcgatgctagcaccggtaccaggaccacccagcagttccggcgccggttttggcgtttagtatg

SEQ ID NO: 27 - DNA, 36 bp, Artificial Sequence; identical to SEQ ID NO: 17
  Primer for NM23 S120G IgG1h noC (modified hinge region of IgG1 without cysteines)

SEQ ID NO: 28 - DNA, 31 bp, Artificial Sequence; identical to SEQ ID NO: 4
  Primer for NM23 S120G IgG1h noC (modified hinge region of IgG1 without cysteines)

SEQ ID NO: 29 - DNA, 32 bp, Artificial Sequence; identical to SEQ ID NO: 3
  Primer for NM23 S120G IgG2a noC  (modified hinge region of IgG2a without cysteines)

SEQ ID NO: 30 - DNA, 66 bp, Artificial Sequence
  Primer for NM23 S120G IgG2a noC  (modified hinge region of IgG2a without cysteines)
tcggaggtttcggaggtttaatagtcggaccaccagtttcatagatccagttctgagcacagctcg

SEQ ID NO: 31 - DNA, 32 bp, Artificial Sequence; identical to SEQ ID NO: 3
  Primer for NM23 S120G IgG2a noC  (modified hinge region of IgG2a without cysteines)

SEQ ID NO: 32 - DNA, 68 bp, Artificial Sequence
  Primer for NM23 S120G IgG2a noC  (modified hinge region of IgG2a without cysteines)
atcgatgctagccggaccacccagcaggttcggagcaggtttcggaggtttcggaggtttaatagtcg

SEQ ID NO: 33 - DNA, 36 bp, Artificial Sequence; identical to SEQ ID NO: 17
  Primer for NM23 S120G IgG2a noC  (modified hinge region of IgG2a without cysteines)

SEQ ID NO: 34 - DNA, 31 bp, Artificial Sequence; identical to SEQ ID NO: 4
  Primer for NM23 S120G IgG2a noC  (modified hinge region of IgG2a without cysteines)

SEQ ID NO: 35 - DNA, 32 bp, Artificial Sequence; identical to SEQ ID NO: 3
  Primer for NM23 S120G  IgG1h/IgG2ah noC (modified hinge region of IgG1 and  IgG2a without cysteines)

SEQ ID NO: 36 - DNA, 67 bp, Artificial Sequence; identical to SEQ ID NO: 24
  Primer for NM23 S120G  IgG1h/IgG2ah noC (modified hinge region of IgG1 and  IgG2a without cysteines)

SEQ ID NO: 37 - DNA, 32 bp, Artificial Sequence; identical to SEQ ID NO: 3
  Primer for NM23 S120G  IgG1h/IgG2ah noC (modified hinge region of IgG1 and  IgG2a without cysteines)

SEQ ID NO: 38 - DNA, 67 bp, Artificial Sequence
  Primer for NM23 S120G  IgG1h/IgG2ah noC (modified hinge region of IgG1 and  IgG2a without cysteines)
tcggaccaccagtaccggtaccaggaccacccagcagttccggcgccggttttggcggtttagtatg

SEQ ID NO: 39 - DNA, 32 bp, Artificial Sequence; identical to SEQ ID NO: 3
  Primer for NM23 S120G  IgG1h/IgG2ah noC (modified hinge region of IgG1 and  IgG2a without cysteines)

SEQ ID NO: 40 - DNA, 66 bp, Artificial Sequence
  Primer for NM23 S120G  IgG1h/IgG2ah noC (modified hinge region of IgG1 and  IgG2a without cysteines)
tcggagcaggtttcggaggtttcggaggtttaatagtcggaccaccagtaccggtaccaggaccac

SEQ ID NO: 41 - DNA, 32 bp, Artificial Sequence; identical to SEQ ID NO: 3
  Primer for NM23 S120G  IgG1h/IgG2ah noC (modified hinge region of IgG1 and  IgG2a without cysteines)

SEQ ID NO: 42 - DNA, 56 bp, Artificial Sequence
  Primer for NM23 S120G  IgG1h/IgG2ah noC (modified hinge region of IgG1 and  IgG2a without cysteines)
atcgatgctagccggaccacccagcaggttcggagcaggtttcggaggtttcggag

SEQ ID NO: 43 - DNA, 36 bp, Artificial Sequence; identical to SEQ ID NO: 17
  Primer for NM23 S120G  IgG1h/IgG2ah noC (modified hinge region of IgG1 and  IgG2a without cysteines)

SEQ ID NO: 44 - DNA, 31 bp, Artificial Sequence; identical to SEQ ID NO: 4
  Primer for NM23 S120G  IgG1h/IgG2ah noC (modified hinge region of IgG1 and  IgG2a without cysteines)

SEQ ID NO: 45 - DNA, 32 bp, Artificial Sequence; identical to SEQ ID NO: 3
  Primer for NM23 S120G-IgG1 Fc (NM23 fused to the Fc region antibody)

SEQ ID NO: 46 - DNA, 31 bp, Artificial Sequence; identical to SEQ ID NO: 4
  Primer for NM23 S120G-IgG1 Fc (NM23 fused to the Fc region antibody)

SEQ ID NO: 47 - DNA, 43 bp, Artificial Sequence
  Primer for NM23 S120G-IgG1 Fc (NM23 fused to the Fc region antibody)
attgtgctcgagggttgtaagccttgcatatgtacagtcccag

SEQ ID NO: 48 - DNA, 44 bp, Artificial Sequence
  Primer for NM23 S120G-IgG1 Fc (NM23 fused to the Fc region antibody)
gcactactcgagtttaccaggagagtgggagaggctcttctcag

SEQ ID NO: 49 - DNA, 32 bp, Artificial Sequence; identical to SEQ ID NO: 3
  Primer for NM23 S120G IgG1h (NM23 fused to the hinge region of IgG1)

SEQ ID NO: 50 - DNA, 86 bp, Artificial Sequence
  Primer for NM23 S120G IgG1h (NM23 fused to the hinge region of IgG1)
atcgatctcgagaccaacacaaatacacggtttacaaccagaatcacgtggcaccggttcatagatccagttctgagcacagctcg

SEQ ID NO: 51 - DNA, 32 bp, Artificial Sequence; identical to SEQ ID NO: 3
  Primer for NM23 S120G IgG2ah( NM23 fused to the hinge region of IgG2a)

SEQ ID NO: 52 - DNA, 89 bp, Artificial Sequence
  Primer for NM23 S120G IgG2ah( NM23 fused to the hinge region of IgG2a)
atcgatctcgagacctggacatttacacggtggacacggtttaatggtcggaccacgcggttcatagatccagttctgagcacagctcg

SEQ ID NO: 53 - protein, 10 aa, Artificial Sequence
  Linker
GGGGSGGGGS

SEQ ID NO: 54 - protein, 15 aa, Artificial Sequence
  Linker
GGGGSGGGGSGGGGS

SEQ ID NO: 55 - protein, 21 aa, Artificial Sequence
  Linker
DKTHTKPPKPAPELLGGPGTG

SEQ ID NO: 56 - protein, 22 aa, Artificial Sequence
  Linker
TGGPTIKPPKPPKPAPNLLGGP

SEQ ID NO: 57 - protein, 43 aa, Artificial Sequence
  Linker
DKTHTKPPKPAPELLGGPGTGTGGPTIKPPKPPKPAPNLLGGP

SEQ ID NO: 58 - protein, 11 aa, Artificial Sequence
  Linker
GCKPCICTVPE

SEQ ID NO: 59 - protein, 15 aa, Artificial Sequence
  Linker
PVPRDSGCKPCICVG

SEQ ID NO: 60 - protein, 16 aa, Artificial Sequence
  Linker
PRGPTIKPCPPCKCPG

SEQ ID NO: 61 - DNA, 483 bp, Artificial Sequence
  NM23 S120G cloned between NdeI and XhoI
atggccaactgtgagcgtaccttcattgcgatcaaaccagatggggtccagcggggtcttgtgggagagattatcaagcgttttgagcagaaaggattccgccttgttggtctgaaattcatgcaagcttccgaagatcttctcaaggaacactacgttgacctgaaggaccgtccattctttgccggcctggtgaaatacatgcactcagggccggtagttgccatggtctgggaggggctgaatgtggtgaagacgggccgagtcatgctcggggagaccaaccctgcagactccaagcctgggaccatccgtggagacttctgcatacaagttggcaggaacattatacatggcggtgattctgtggagagtgcagagaaggagatcggcttgtggtttcaccctgaggaactggtagattacacgagctgtgctcagaactggatctatgaactcgagcaccaccaccaccaccactga

SEQ ID NO: 62 - protein, 160 aa, Artificial Sequence
  NM23 S120G cloned between NdeI and XhoI with histidine tag at the C-terminus
MANCERTFIAIKPDGVQRGLVGEIIKRFEQKGFRLVGLKFMQASEDLLKEHYVDLKDRPFFAGLVKYMHSGPVVAMVWEGLNVVKTGRVMLGETNPADSKPGTIRGDFCIQVGRNIIHGGDSVESAEKEIGLWFHPEELVDYTSCAQNWIYELEHHHHHH

SEQ ID NO: 63 - DNA, 483 bp, Artificial Sequence
  NM23 S120G alternate clone cloned between NdeI and AgeI
atggccaactgtgagcgtaccttcattgcgatcaaaccagatggggtccagcggggtcttgtgggagagattatcaagcgttttgagcagaaaggattccgccttgttggtctgaaattcatgcaagcttccgaagatcttctcaaggaacactacgttgacctgaaggaccgtccattctttgccggcctggtgaaatacatgcactcagggccggtagttgccatggtctgggaggggctgaatgtggtgaagacgggccgagtcatgctcggggagaccaaccctgcagactccaagcctgggaccatccgtggagacttctgcatacaagttggcaggaacattatacatggcggtgattctgtggagagtgcagagaaggagatcggcttgtggtttcaccctgaggaactggtagattacacgagctgtgctcagaactggatctatgaaaccggtcaccaccaccaccaccactga

SEQ ID NO: 64 - protein, 160 aa, Artificial Sequence
  NM23 S120G alternate clone cloned between NdeI and AgeI with histidine tag at the C-terminus
MANCERTFIAIKPDGVQRGLVGEIIKRFEQKGFRLVGLKFMQASEDLLKEHYVDLKDRPFFAGLVKYMHSGPVVAMVWEGLNVVKTGRVMLGETNPADSKPGTIRGDFCIQVGRNIIHGGDSVESAEKEIGLWFHPEELVDYTSCAQNWIYETGHHHHHH

SEQ ID NO: 65 - DNA, 483 bp, Artificial Sequence
  NM23 P96S cloned between NdeI and AgeI
atggccaactgtgagcgtaccttcattgcgatcaaaccagatggggtccagcggggtcttgtgggagagattatcaagcgttttgagcagaaaggattccgccttgttggtctgaaattcatgcaagcttccgaagatcttctcaaggaacactacgttgacctgaaggaccgtccattctttgccggcctggtgaaatacatgcactcagggccggtagttgccatggtctgggaggggctgaatgtggtgaagacgggccgagtcatgctcggggagaccaactctgcagactccaagcctgggaccatccgtggagacttctgcatacaagttggcaggaacattatacatggcagtgattctgtggagagtgcagagaaggagatcggcttgtggtttcaccctgaggaactggtagattacacgagctgtgctcagaactggatctatgaaaccggtcaccaccaccaccaccactga

SEQ ID NO: 66 - protein, 160 aa, Artificial Sequence
  NM23 P96S cloned between NdeI and AgeI with histidine tag at the C-terminus
MANCERTFIAIKPDGVQRGLVGEIIKRFEQKGFRLVGLKFMQASEDLLKEHYVDLKDRPFFAGLVKYMHSGPVVAMVWEGLNVVKTGRVMLGETNSADSKPGTIRGDFCIQVGRNIIHGSDSVESAEKEIGLWFHPEELVDYTSCAQNWIYETGHHHHHH

SEQ ID NO: 67 - DNA, 483 bp, Artificial Sequence
  NM23 P96S/S120G cloned between NdeI and AgeI
atggccaactgtgagcgtaccttcattgcgatcaaaccagatggggtccagcggggtcttgtgggagagattatcaagcgttttgagcagaaaggattccgccttgttggtctgaaattcatgcaagcttccgaagatcttctcaaggaacactacgttgacctgaaggaccgtccattctttgccggcctggtgaaatacatgcactcagggccggtagttgccatggtctgggaggggctgaatgtggtgaagacgggccgagtcatgctcggggagaccaactctgcagactccaagcctgggaccatccgtggagacttctgcatacaagttggcaggaacattatacatggcggtgattctgtggagagtgcagagaaggagatcggcttgtggtttcaccctgaggaactggtagattacacgagctgtgctcagaactggatctatgaaaccggtcaccaccaccaccaccactga

SEQ ID NO: 68 - protein, 160 aa, Artificial Sequence
  NM23 P96S/S120G cloned between NdeI and AgeI with histidine tag at the C-terminus
MANCERTFIAIKPDGVQRGLVGEIIKRFEQKGFRLVGLKFMQASEDLLKEHYVDLKDRPFFAGLVKYMHSGPVVAMVWEGLNVVKTGRVMLGETNSADSKPGTIRGDFCIQVGRNIIHGGDSVESAEKEIGLWFHPEELVDYTSCAQNWIYETGHHHHHH

SEQ ID NO: 69 - DNA, 480 bp, Artificial Sequence
  NM23 P96S Delta C1 cloned between NdeI and AgeI
atggccaactgtgagcgtaccttcattgcgatcaaaccagatggggtccagcggggtcttgtgggagagattatcaagcgttttgagcagaaaggattccgccttgttggtctgaaattcatgcaagcttccgaagatcttctcaaggaacactacgttgacctgaaggaccgtccattctttgccggcctggtgaaatacatgcactcagggccggtagttgccatggtctgggaggggctgaatgtggtgaagacgggccgagtcatgctcggggagaccaactctgcagactccaagcctgggaccatccgtggagacttctgcatacaagttggcaggaacattatacatggcagtgattctgtggagagtgcagagaaggagatcggcttgtggtttcaccctgaggaactggtagattacacgagctgtgctcagaactggatctataccggtcaccaccaccaccaccactga

SEQ ID NO: 70 - protein, 159 aa, Artificial Sequence
  NM23 P96S Delta C1 cloned between NdeI and AgeI with histidine tag at the C-terminus
MANCERTFIAIKPDGVQRGLVGEIIKRFEQKGFRLVGLKFMQASEDLLKEHYVDLKDRPFFAGLVKYMHSGPVVAMVWEGLNVVKTGRVMLGETNSADSKPGTIRGDFCIQVGRNIIHGSDSVESAEKEIGLWFHPEELVDYTSCAQNWIYTGHHHHHH

SEQ ID NO: 71 - DNA, 477 bp, Artificial Sequence
  NM23 P96S Delta C2 cloned between NdeI and AgeI
atggccaactgtgagcgtaccttcattgcgatcaaaccagatggggtccagcggggtcttgtgggagagattatcaagcgttttgagcagaaaggattccgccttgttggtctgaaattcatgcaagcttccgaagatcttctcaaggaacactacgttgacctgaaggaccgtccattctttgccggcctggtgaaatacatgcactcagggccggtagttgccatggtctgggaggggctgaatgtggtgaagacgggccgagtcatgctcggggagaccaactctgcagactccaagcctgggaccatccgtggagacttctgcatacaagttggcaggaacattatacatggcagtgattctgtggagagtgcagagaaggagatcggcttgtggtttcaccctgaggaactggtagattacacgagctgtgctcagaactggatcaccggtcaccaccaccaccaccactga

SEQ ID NO: 72 - protein, 158 aa, Artificial Sequence
  NM23 P96S Delta C2 cloned between NdeI and AgeI with histidine tag at the C-terminus
MANCERTFIAIKPDGVQRGLVGEIIKRFEQKGFRLVGLKFMQASEDLLKEHYVDLKDRPFFAGLVKYMHSGPVVAMVWEGLNVVKTGRVMLGETNSADSKPGTIRGDFCIQVGRNIIHGSDSVESAEKEIGLWFHPEELVDYTSCAQNWITGHHHHHH

SEQ ID NO: 73 - DNA, 465 bp, Artificial Sequence
  NM23 P96S Delta C6 cloned between NdeI and AgeI
atggccaactgtgagcgtaccttcattgcgatcaaaccagatggggtccagcggggtcttgtgggagagattatcaagcgttttgagcagaaaggattccgccttgttggtctgaaattcatgcaagcttccgaagatcttctcaaggaacactacgttgacctgaaggaccgtccattctttgccggcctggtgaaatacatgcactcagggccggtagttgccatggtctgggaggggctgaatgtggtgaagacgggccgagtcatgctcggggagaccaactctgcagactccaagcctgggaccatccgtggagacttctgcatacaagttggcaggaacattatacatggcagtgattctgtggagagtgcagagaaggagatcggcttgtggtttcaccctgaggaactggtagattacacgagctgtgctaccggtcaccaccaccaccaccactga

SEQ ID NO: 74 - protein, 154 aa, Artificial Sequence
  NM23 P96S Delta C6 cloned between NdeI and AgeI with histidine tag at the C-terminus
MANCERTFIAIKPDGVQRGLVGEIIKRFEQKGFRLVGLKFMQASEDLLKEHYVDLKDRPFFAGLVKYMHSGPVVAMVWEGLNVVKTGRVMLGETNSADSKPGTIRGDFCIQVGRNIIHGSDSVESAEKEIGLWFHPEELVDYTSCATGHHHHHH

SEQ ID NO: 75 - DNA, 480 bp, Artificial Sequence
  NM23 P96S Delta C1 /S120G cloned between NdeI and AgeI
atggccaactgtgagcgtaccttcattgcgatcaaaccagatggggtccagcggggtcttgtgggagagattatcaagcgttttgagcagaaaggattccgccttgttggtctgaaattcatgcaagcttccgaagatcttctcaaggaacactacgttgacctgaaggaccgtccattctttgccggcctggtgaaatacatgcactcagggccggtagttgccatggtctgggaggggctgaatgtggtgaagacgggccgagtcatgctcggggagaccaactctgcagactccaagcctgggaccatccgtggagacttctgcatacaagttggcaggaacattatacatggcggtgattctgtggagagtgcagagaaggagatcggcttgtggtttcaccctgaggaactggtagattacacgagctgtgctcagaactggatctataccggtcaccaccaccaccaccactga

SEQ ID NO: 76 - protein, 159 aa, Artificial Sequence
  NM23 P96S Delta C1 /S120G cloned between NdeI and AgeI with histidine tag at the C-terminus
MANCERTFIAIKPDGVQRGLVGEIIKRFEQKGFRLVGLKFMQASEDLLKEHYVDLKDRPFFAGLVKYMHSGPVVAMVWEGLNVVKTGRVMLGETNSADSKPGTIRGDFCIQVGRNIIHGGDSVESAEKEIGLWFHPEELVDYTSCAQNWIYTGHHHHHH

SEQ ID NO: 77 - DNA, 477 bp, Artificial Sequence
  NM23 P96S Delta C2 /S120G cloned between NdeI and AgeI
atggccaactgtgagcgtaccttcattgcgatcaaaccagatggggtccagcggggtcttgtgggagagattatcaagcgttttgagcagaaaggattccgccttgttggtctgaaattcatgcaagcttccgaagatcttctcaaggaacactacgttgacctgaaggaccgtccattctttgccggcctggtgaaatacatgcactcagggccggtagttgccatggtctgggaggggctgaatgtggtgaagacgggccgagtcatgctcggggagaccaactctgcagactccaagcctgggaccatccgtggagacttctgcatacaagttggcaggaacattatacatggcggtgattctgtggagagtgcagagaaggagatcggcttgtggtttcaccctgaggaactggtagattacacgagctgtgctcagaactggatcaccggtcaccaccaccaccaccactga

SEQ ID NO: 78 - protein, 158 aa, Artificial Sequence
  NM23 P96S Delta C2 /S120G cloned between NdeI and AgeI with histidine tag at the C-terminus
MANCERTFIAIKPDGVQRGLVGEIIKRFEQKGFRLVGLKFMQASEDLLKEHYVDLKDRPFFAGLVKYMHSGPVVAMVWEGLNVVKTGRVMLGETNSADSKPGTIRGDFCIQVGRNIIHGGDSVESAEKEIGLWFHPEELVDYTSCAQNWITGHHHHHH

SEQ ID NO: 79 - DNA, 465 bp, Artificial Sequence
  NM23 P96S Delta C6 /S120G cloned between NdeI and AgeI
atggccaactgtgagcgtaccttcattgcgatcaaaccagatggggtccagcggggtcttgtgggagagattatcaagcgttttgagcagaaaggattccgccttgttggtctgaaattcatgcaagcttccgaagatcttctcaaggaacactacgttgacctgaaggaccgtccattctttgccggcctggtgaaatacatgcactcagggccggtagttgccatggtctgggaggggctgaatgtggtgaagacgggccgagtcatgctcggggagaccaactctgcagactccaagcctgggaccatccgtggagacttctgcatacaagttggcaggaacattatacatggcggtgattctgtggagagtgcagagaaggagatcggcttgtggtttcaccctgaggaactggtagattacacgagctgtgctaccggtcaccaccaccaccaccactga

SEQ ID NO: 80 - protein, 154 aa, Artificial Sequence
  NM23 P96S Delta C6 /S120G cloned between NdeI and AgeI with histidine tag at the C-terminus
MANCERTFIAIKPDGVQRGLVGEIIKRFEQKGFRLVGLKFMQASEDLLKEHYVDLKDRPFFAGLVKYMHSGPVVAMVWEGLNVVKTGRVMLGETNSADSKPGTIRGDFCIQVGRNIIHGGDSVESAEKEIGLWFHPEELVDYTSCATGHHHHHH

SEQ ID NO: 81 - DNA, 30 bp, Artificial Sequence
  GS2 linker
ggcggtggcggatccggcggtggcggatcc

SEQ ID NO: 82 - protein, 10 aa, Artificial Sequence
  GS2 linker
GGGGSGGGGS

SEQ ID NO: 83 - DNA, 45 bp, Artificial Sequence
  GS3 linker
ggcggtggcggatccggcggtggcggatccggcggtggcggatcc

SEQ ID NO: 84 - protein, 15 aa, Artificial Sequence
  GS3 linker
GGGGSGGGGSGGGGS

SEQ ID NO: 85 - DNA, 63 bp, Artificial Sequence
  IgG1h no C linker (modified hinge portion of an Fc region of an antibody)
gataaaacccatactaaaccgccaaaaccggcgccggaactgctgggtggtcctggtaccggt

SEQ ID NO: 86 - protein, 21 aa, Artificial Sequence
  IgG1h no C linker (modified hinge portion of an Fc region of an antibody)
DKTHTKPPKPAPELLGGPGTG

SEQ ID NO: 87 - DNA, 66 bp, Artificial Sequence
  IgG2ah no C linker (modified hinge portion of an Fc region of an antibody)
actggtggtccgactattaaacctccgaaacctccgaaacctgctccgaacctgctgggtggtccg

SEQ ID NO: 88 - protein, 22 aa, Artificial Sequence
  IgG2ah no C linker (modified hinge portion of an Fc region of an antibody)
TGGPTIKPPKPPKPAPNLLGGP

SEQ ID NO: 89 - DNA, 129 bp, Artificial Sequence
  IgG1h/IgG2ah no C linker (combined hinge portions of two Fc regions of two different isotype antibodies
gataaaacccatactaaaccgccaaaaccggcgccggaactgctgggtggtcctggtaccggtactggtggtccgactattaaacctccgaaacctccgaaacctgctccgaacctgctgggtggtccg

SEQ ID NO: 90 - protein, 43 aa, Artificial Sequence; identical to SEQ ID NO: 57
  IgG1h/IgG2ah no C linker (combined hinge portions of two Fc regions of two different isotype antibodies

SEQ ID NO: 91 - DNA, 1155 bp, Artificial Sequence
  NM23 S120G IgG1Fc (NM23-X connected to the Fc region of an antibody )
atggccaactgtgagcgtaccttcattgcgatcaaaccagatggggtccagcggggtcttgtgggagagattatcaagcgttttgagcagaaaggattccgccttgttggtctgaaattcatgcaagcttccgaagatcttctcaaggaacactacgttgacctgaaggaccgtccattctttgccggcctggtgaaatacatgcactcagggccggtagttgccatggtctgggaggggctgaatgtggtgaagacgggccgagtcatgctcggggagaccaaccctgcagactccaagcctgggaccatccgtggagacttctgcatacaagttggcaggaacattatacatggcggtgattctgtggagagtgcagagaaggagatcggcttgtggtttcaccctgaggaactggtagattacacgagctgtgctcagaactggatctatgaactcgagggttgtaagccttgcatatgtacagtcccagaagtatcatctgtcttcatcttccccccaaagcccaaggatgtgctcaccattactctgactcctaaggtcacgtgtgttgtggtagacatcagcaaggatgatcccgaggtccagttcagctggtttgtagatgatgtggaggtgcacacagctcagacgcaaccccgggaggagcagttcaacagcactttccgctcagtcagtgaacttcccatcatgcaccaggactggctcaatggcaaggagttcaaatgcagggtcaacagtgcagctttccctgcccccatcgagaaaaccatctccaaaaccaaaggcagaccgaaggctccacaggtgtacaccattccacctcccaaggagcagatggccaaggataaagtcagtctgacctgcatgataacagacttcttccctgaagacattactgtggagtggcagtggaatgggcagccagcggagaactacaagaacactcagcccatcatggacacagatggctcttacttcgtctacagcaagctcaatgtgcagaagagcaactgggaggcaggaaatactttcacctgctctgtgttacatgagggcctgcacaaccaccatactgagaagagcctctcccactctcctggtaaactcgagcaccaccaccaccaccactga

SEQ ID NO: 92 - protein, 384 aa, Artificial Sequence
  NM23 S120G IgG1Fc (NM23-X connected to the Fc region of an antibody) with histidine tag at the C-terminus
MANCERTFIAIKPDGVQRGLVGEIIKRFEQKGFRLVGLKFMQASEDLLKEHYVDLKDRPFFAGLVKYMHSGPVVAMVWEGLNVVKTGRVMLGETNPADSKPGTIRGDFCIQVGRNIIHGGDSVESAEKEIGLWFHPEELVDYTSCAQNWIYELEGCKPCICTVPEVSSVFIFPPKPKDVLTITLTPKVTCVVVDISKDDPEVQFSWFVDDVEVHTAQTQPREEQFNSTFRSVSELPIMHQDWLNGKEFKCRVNSAAFPAPIEKTISKTKGRPKAPQVYTIPPPKEQMAKDKVSLTCMITDFFPEDITVEWQWNGQPAENYKNTQPIMDTDGSYFVYSKLNVQKSNWEAGNTFTCSVLHEGLHNHHTEKSLSHSPGKLEHHHHHH

SEQ ID NO: 93 - DNA, 528 bp, Artificial Sequence
  NM23 S120G IgG1h (NM23-X connected to only modified hinge portion of the Fc region of an antibody )
atggccaactgtgagcgtaccttcattgcgatcaaaccagatggggtccagcggggtcttgtgggagagattatcaagcgttttgagcagaaaggattccgccttgttggtctgaaattcatgcaagcttccgaagatcttctcaaggaacactacgttgacctgaaggaccgtccattctttgccggcctggtgaaatacatgcactcagggccggtagttgccatggtctgggaggggctgaatgtggtgaagacgggccgagtcatgctcggggagaccaaccctgcagactccaagcctgggaccatccgtggagacttctgcatacaagttggcaggaacattatacatggcggtgattctgtggagagtgcagagaaggagatcggcttgtggtttcaccctgaggaactggtagattacacgagctgtgctcagaactggatctatgaaccggtgccacgtgattctggttgtaaaccgtgtatttgtgttggtctcgagcaccaccaccaccaccactga

SEQ ID NO: 94 - protein, 175 aa, Artificial Sequence
  NM23 S120G IgG1h (NM23-X connected to only modified hinge portion of the Fc region of an antibody ) with histidine tag at the C-terminus
MANCERTFIAIKPDGVQRGLVGEIIKRFEQKGFRLVGLKFMQASEDLLKEHYVDLKDRPFFAGLVKYMHSGPVVAMVWEGLNVVKTGRVMLGETNPADSKPGTIRGDFCIQVGRNIIHGGDSVESAEKEIGLWFHPEELVDYTSCAQNWIYEPVPRDSGCKPCICVGLEHHHHHH

SEQ ID NO: 95 - DNA, 531 bp, Artificial Sequence
  NM23 S120G IgG2ah (NM23-X connected to only modified hinge portion of the Fc region of an antibody )
atggccaactgtgagcgtaccttcattgcgatcaaaccagatggggtccagcggggtcttgtgggagagattatcaagcgttttgagcagaaaggattccgccttgttggtctgaaattcatgcaagcttccgaagatcttctcaaggaacactacgttgacctgaaggaccgtccattctttgccggcctggtgaaatacatgcactcagggccggtagttgccatggtctgggaggggctgaatgtggtgaagacgggccgagtcatgctcggggagaccaaccctgcagactccaagcctgggaccatccgtggagacttctgcatacaagttggcaggaacattatacatggcggtgattctgtggagagtgcagagaaggagatcggcttgtggtttcaccctgaggaactggtagattacacgagctgtgctcagaactggatctatgaaccgcgtggtccgaccattaaaccgtgtccaccgtgtaaatgtccaggtctcgagcaccaccaccaccaccactga

SEQ ID NO: 96 - protein, 176 aa, Artificial Sequence
  NM23 S120G IgG2ah (NM23-X connected to only modified hinge portion of the Fc region of an antibody ) with histidine tag at the C-terminus
MANCERTFIAIKPDGVQRGLVGEIIKRFEQKGFRLVGLKFMQASEDLLKEHYVDLKDRPFFAGLVKYMHSGPVVAMVWEGLNVVKTGRVMLGETNPADSKPGTIRGDFCIQVGRNIIHGGDSVESAEKEIGLWFHPEELVDYTSCAQNWIYEPRGPTIKPCPPCKCPGLEHHHHHH

SEQ ID NO: 97 - DNA, 459 bp, Homo sapiens
atggccaactgtgagcgtaccttcattgcgatcaaaccagatggggtccagcggggtcttgtgggagagattatcaagcgttttgagcagaaaggattccgccttgttggtctgaaattcatgcaagcttccgaagatcttctcaaggaacactacgttgacctgaaggaccgtccattctttgccggcctggtgaaatacatgcactcagggccggtagttgccatggtctgggaggggctgaatgtggtgaagacgggccgagtcatgctcggggagaccaaccctgcagactccaagcctgggaccatccgtggagacttctgcatacaagttggcaggaacattatacatggcagtgattctgtggagagtgcagagaaggagatcggcttgtggtttcaccctgaggaactggtagattacacgagctgtgctcagaactggatctatgaatga

SEQ ID NO: 98 - protein, 152 aa, Homo sapiens
MANCERTFIAIKPDGVQRGLVGEIIKRFEQKGFRLVGLKFMQASEDLLKEHYVDLKDRPFFAGLVKYMHSGPVVAMVWEGLNVVKTGRVMLGETNPADSKPGTIRGDFCIQVGRNIIHGSDSVESAEKEIGLWFHPEELVDYTSCAQNWIYE

SEQ ID NO: 99 - DNA, 459 bp, Mus musculus
atggccaacagtgagcgcaccttcattgccatcaagcctgatggggtccagcgggggctggtgggcgagatcatcaagcggttcgagcagaaggggttccgccttgttggtctgaagtttctgcaggcttcagaggaccttctcaaggagcactacactgacctgaaggaccgccccttctttactggcctggtgaaatacatgcactcaggaccagtggttgctatggtctgggagggtctgaatgtggtgaagacaggccgcgtgatgcttggagagaccaaccccgcagactctaagcctgggaccatacgaggagacttctgcatccaagttggcaggaacatcattcatggcagcgattctgtaaagagcgcagagaaggagatcagcttgtggtttcagcctgaggagctggtggagtacaagagctgtgcgcagaactggatctatgagtga

SEQ ID NO: 100 - protein, 152 aa, Mus musculus
MANSERTFIAIKPDGVQRGLVGEIIKRFEQKGFRLVGLKFLQASEDLLKEHYTDLKDRPFFTGLVKYMHSGPVVAMVWEGLNVVKTGRVMLGETNPADSKPGTIRGDFCIQVGRNIIHGSDSVKSAEKEISLWFQPEELVEYKSCAQNWIYE

SEQ ID NO: 101 - DNA, 459 bp, Homo sapiens
atggccaacctggagcgcaccttcatcgccatcaagccggacggcgtgcagcgcggcctggtgggcgagatcatcaagcgcttcgagcagaagggattccgcctcgtggccatgaagttcctccgggcctctgaagaacacctgaagcagcactacattgacctgaaagaccgaccattcttccctgggctggtgaagtacatgaactcagggccggttgtggccatggtctgggaggggctgaacgtggtgaagacaggccgagtgatgcttggggagaccaatccagcagattcaaagccaggcaccattcgtggggacttctgcattcaggttggcaggaacatcattcatggcagtgattcagtaaaaagtgctgaaaaagaaatcagcctatggtttaagcctgaagaactggttgactacaagtcttgtgctcatgactgggtctatgaataa

SEQ ID NO: 102 - protein, 152 aa, Homo sapiens
MANLERTFIAIKPDGVQRGLVGEIIKRFEQKGFRLVAMKFLRASEEHLKQHYIDLKDRPFFPGLVKYMNSGPVVAMVWEGLNVVKTGRVMLGETNPADSKPGTIRGDFCIQVGRNIIHGSDSVKSAEKEISLWFKPEELVDYKSCAHDWVYE

SEQ ID NO: 103 - DNA, 459 bp, Mus musculus
atggccaacctcgagcgtaccttcattgccatcaagccagatggcgtgcagcgcggcctggtgggcgagatcatcaaacggttcgagcagaaggggttccgcctggtggccatgaagttccttcgggcctctgaagaacacctgaagcagcattacatcgacctgaaagaccgtcctttcttcccggggctggtgaagtacatgaactcggggcccgtggtggccatggtctgggaggggctcaatgtggtgaaaacgggccgagtgatgctgggggagaccaatccagctgattcaaaaccaggcaccatccgtggggatttctgcattcaagttggcaggaacatcattcatggcagtgattcagtggagagtgctgagaaagagatccatctgtggtttaagcccgaagaactgatcgactacaagtcttgtgcccatgactgggtgtacgagtag

SEQ ID NO: 104 - protein, 152 aa, Mus musculus
MANLERTFIAIKPDGVQRGLVGEIIKRFEQKGFRLVAMKFLRASEEHLKQHYIDLKDRPFFPGLVKYMNSGPVVAMVWEGLNVVKTGRVMLGETNPADSKPGTIRGDFCIQVGRNIIHGSDSVESAEKEIHLWFKPEELIDYKSCAHDWVYE

SEQ ID NO: 105 - DNA, 1131 bp, Homo sapiens
atgaatcatagtgaaagattcgttttcattgcagagtggtatgatccaaatgcttcacttcttcgacgttatgagcttttattttacccaggggatggatctgttgaaatgcatgatgtaaagaatcatcgcacctttttaaagcggaccaaatatgataacctgcacttggaagatttatttataggcaacaaagtgaatgtcttttctcgacaactggtattaattgactatggggatcaatatacagctcgccagctgggcagtaggaaagaaaaaacgctagccctaattaaaccagatgcaatatcaaaggctggagaaataattgaaataataaacaaagctggatttactataaccaaactcaaaatgatgatgctttcaaggaaagaagcattggattttcatgtagatcaccagtcaagaccctttttcaatgagctgatccagtttattacaactggtcctattattgccatggagattttaagagatgatgctatatgtgaatggaaaagactgctgggacctgcaaactctggagtggcacgcacagatgcttctgaaagcattagagccctctttggaacagatggcataagaaatgcagcgcatggccctgattcttttgcttctgcggccagagaaatggagttgttttttccttcaagtggaggttgtgggccggcaaacactgctaaatttactaattgtacctgttgcattgttaaaccccatgctgtcagtgaaggactgttgggaaagatcctgatggctatccgagatgcaggttttgaaatctcagctatgcagatgttcaatatggatcgggttaatgttgaggaattctatgaagtttataaaggagtagtgaccgaatatcatgacatggtgacagaaatgtattctggcccttgtgtagcaatggagattcaacagaataatgctacaaagacatttcgagaattttgtggacctgctgatcctgaaattgcccggcatttacgccctggaactctcagagcaatctttggtaaaactaagatccagaatgctgttcactgtactgatctgccagaggatggcctattagaggttcaatacttcttcaagatcttggataattag

SEQ ID NO: 106 - protein, 376 aa, Homo sapiens
MNHSERFVFIAEWYDPNASLLRRYELLFYPGDGSVEMHDVKNHRTFLKRTKYDNLHLEDLFIGNKVNVFSRQLVLIDYGDQYTARQLGSRKEKTLALIKPDAISKAGEIIEIINKAGFTITKLKMMMLSRKEALDFHVDHQSRPFFNELIQFITTGPIIAMEILRDDAICEWKRLLGPANSGVARTDASESIRALFGTDGIRNAAHGPDSFASAAREMELFFPSSGGCGPANTAKFTNCTCCIVKPHAVSEGLLGKILMAIRDAGFEISAMQMFNMDRVNVEEFYEVYKGVVTEYHDMVTEMYSGPCVAMEIQQNNATKTFREFCGPADPEIARHLRPGTLRAIFGKTKIQNAVHCTDLPEDGLLEVQYFFKILDN

SEQ ID NO: 107 - DNA, 1131 bp, Artificial Sequence
  Human NM23-H7-1 sequence optimized for E. coli expression
atgaatcactccgaacgctttgtttttatcgccgaatggtatgacccgaatgcttccctgctgcgccgctacgaactgctgttttatccgggcgatggtagcgtggaaatgcatgacgttaaaaatcaccgtacctttctgaaacgcacgaaatatgataatctgcatctggaagacctgtttattggcaacaaagtcaatgtgttctctcgtcagctggtgctgatcgattatggcgaccagtacaccgcgcgtcaactgggtagtcgcaaagaaaaaacgctggccctgattaaaccggatgcaatctccaaagctggcgaaattatcgaaattatcaacaaagcgggtttcaccatcacgaaactgaaaatgatgatgctgagccgtaaagaagccctggattttcatgtcgaccaccagtctcgcccgtttttcaatgaactgattcaattcatcaccacgggtccgattatcgcaatggaaattctgcgtgatgacgctatctgcgaatggaaacgcctgctgggcccggcaaactcaggtgttgcgcgtaccgatgccagtgaatccattcgcgctctgtttggcaccgatggtatccgtaatgcagcacatggtccggactcattcgcatcggcagctcgtgaaatggaactgtttttcccgagctctggcggttgcggtccggcaaacaccgccaaatttaccaattgtacgtgctgtattgtcaaaccgcacgcagtgtcagaaggcctgctgggtaaaattctgatggcaatccgtgatgctggctttgaaatctcggccatgcagatgttcaacatggaccgcgttaacgtcgaagaattctacgaagtttacaaaggcgtggttaccgaatatcacgatatggttacggaaatgtactccggtccgtgcgtcgcgatggaaattcagcaaaacaatgccaccaaaacgtttcgtgaattctgtggtccggcagatccggaaatcgcacgtcatctgcgtccgggtaccctgcgcgcaatttttggtaaaacgaaaatccagaacgctgtgcactgtaccgatctgccggaagacggtctgctggaagttcaatactttttcaaaattctggataattag

SEQ ID NO: 108 - protein, 376 aa, Artificial Sequence; identical to SEQ ID NO: 106
  Human NM23-H7-1 sequence optimized for E. coli expression

SEQ ID NO: 109 - DNA, 1023 bp, Homo sapiens
atgcatgatgtaaagaatcatcgcacctttttaaagcggaccaaatatgataacctgcacttggaagatttatttataggcaacaaagtgaatgtcttttctcgacaactggtattaattgactatggggatcaatatacagctcgccagctgggcagtaggaaagaaaaaacgctagccctaattaaaccagatgcaatatcaaaggctggagaaataattgaaataataaacaaagctggatttactataaccaaactcaaaatgatgatgctttcaaggaaagaagcattggattttcatgtagatcaccagtcaagaccctttttcaatgagctgatccagtttattacaactggtcctattattgccatggagattttaagagatgatgctatatgtgaatggaaaagactgctgggacctgcaaactctggagtggcacgcacagatgcttctgaaagcattagagccctctttggaacagatggcataagaaatgcagcgcatggccctgattcttttgcttctgcggccagagaaatggagttgttttttccttcaagtggaggttgtgggccggcaaacactgctaaatttactaattgtacctgttgcattgttaaaccccatgctgtcagtgaaggactgttgggaaagatcctgatggctatccgagatgcaggttttgaaatctcagctatgcagatgttcaatatggatcgggttaatgttgaggaattctatgaagtttataaaggagtagtgaccgaatatcatgacatggtgacagaaatgtattctggcccttgtgtagcaatggagattcaacagaataatgctacaaagacatttcgagaattttgtggacctgctgatcctgaaattgcccggcatttacgccctggaactctcagagcaatctttggtaaaactaagatccagaatgctgttcactgtactgatctgccagaggatggcctattagaggttcaatacttcttcaagatcttggataattga

SEQ ID NO: 110 - protein, 340 aa, Homo sapiens
MHDVKNHRTFLKRTKYDNLHLEDLFIGNKVNVFSRQLVLIDYGDQYTARQLGSRKEKTLALIKPDAISKAGEIIEIINKAGFTITKLKMMMLSRKEALDFHVDHQSRPFFNELIQFITTGPIIAMEILRDDAICEWKRLLGPANSGVARTDASESIRALFGTDGIRNAAHGPDSFASAAREMELFFPSSGGCGPANTAKFTNCTCCIVKPHAVSEGLLGKILMAIRDAGFEISAMQMFNMDRVNVEEFYEVYKGVVTEYHDMVTEMYSGPCVAMEIQQNNATKTFREFCGPADPEIARHLRPGTLRAIFGKTKIQNAVHCTDLPEDGLLEVQYFFKILDN

SEQ ID NO: 111 - DNA, 1188 bp, Mus musculus
atgagagcctgtcagcagggaagaagttccagtttggtttctccatatatggcacccaagaatcagagcgagagattcgctttcattgcagagtggtatgatccaaatgcttcattgctccgacgctatgagctgctgttttaccccacagacggatctgttgaaatgcatgatgtaaagaatcgtcgcaccttcttaaagcggaccaagtatgaggacctgcgcctggaagatctatttataggcaacaaagtcaatgtgttttctcgacagctggtgttgattgactatggggaccaatacacagcccgccagctgggcagcaggaaagagaaaactttagccctgatcaaaccagatgcagtgtcaaaggccggagaaatcattgagatgataaacaaaagtggatttactataaccaaactccgaatgatgactctgacaaggaaagaagcagcggactttcatgtagaccatcactcaagacctttttataacgaactgatccagtttatcacaagtgggcctgttattgccatggagatcttaagagatgacgcgatctgtgagtggaaaaggttgcttggacccgcaaactctgggctatcacggacagatgcccccggaagcatccgagccctctttgggacagatggcgtgagaaatgcagctcacggccctgatacttttgcatctgctgccagagaaatggaattgttttttccttcaagtggaggctgtgggccagcgaacactgctaaatttaccaattgcacctgttgcatcattaagcctcatgctatcagtgaaggaatgttgggaaagattttaatagctattcgggatgcatgctttggaatgtcagcgatacagatgttcaatttggatcgggctaatgttgaagaattctatgaagtctataaaggtgtagtgtctgagtataatgatatggtgacagagctgtgctccggcccttgcgtagcaatagagatccaacagagcaaccctacaaagacatttcgagaattctgcggacctgctgatcctgaaatcgcccggcatttacgacctgagaccctcagggcaatttttggtaaaactaaggttcaaaatgctgttcattgcacggatctgccggaggatgggctcctggaggtccagtatttcttcaagatcttggataattag

SEQ ID NO: 112 - protein, 395 aa, Mus musculus
MRACQQGRSSSLVSPYMAPKNQSERFAFIAEWYDPNASLLRRYELLFYPTDGSVEMHDVKNRRTFLKRTKYEDLRLEDLFIGNKVNVFSRQLVLIDYGDQYTARQLGSRKEKTLALIKPDAVSKAGEIIEMINKSGFTITKLRMMTLTRKEAADFHVDHHSRPFYNELIQFITSGPVIAMEILRDDAICEWKRLLGPANSGLSRTDAPGSIRALFGTDGVRNAAHGPDTFASAAREMELFFPSSGGCGPANTAKFTNCTCCIIKPHAISEGMLGKILIAIRDACFGMSAIQMFNLDRANVEEFYEVYKGVVSEYNDMVTELCSGPCVAIEIQQSNPTKTFREFCGPADPEIARHLRPETLRAIFGKTKVQNAVHCTDLPEDGLLEVQYFFKILDN

SEQ ID NO: 113 - DNA, 834 bp, Mus musculus
atgagagcctgtcagcagggaagaagttccagtttggtttctccatatatggcacccaagaatcagagcgagagattcgctttcattgcagagtggtatgatccaaatgcttcattgctccgacgctatgagctgctgttttaccccacagacggatctgttgaaatgcatgatgtaaagaatcgtcgcaccttcttaaagcggaccaagtatgaggacctgcgcctggaagatctatttataggcaacaaagtcaatgtgttttctcgacagctggtgttgattgactatggggaccaatacacagcccgccagctgggcagcaggaaagagaaaactttagccctgatcaaaccagatgcagtgtcaaaggccggagaaatcattgagatgataaacaaaagtggatttactataaccaaactccgaatgatgactctgacaaggaaagaagcagcggactttcatgtagaccatcactcaagacctttttataacgaactgatccagtttatcacaagtgggcctgttattgccatggagatcttaagagatgacgcgatctgtgagtggaaaaggttgcttggacccgcaaactctgggctatcacggacagatgcccccggaagcatccgagccctctttgggacagatggcgtgagaaatgcagctcacggccctgatacttttgcatctgctgccagagaaatggaattgttttttccttcaagtggaggctgtgggccagcgaacactgctaaatttaccaattgcacctgttgcatcattaagcctcatgctatcagtgaagatttatttattcattatatgtaa

SEQ ID NO: 114 - protein, 277 aa, Mus musculus
MRACQQGRSSSLVSPYMAPKNQSERFAFIAEWYDPNASLLRRYELLFYPTDGSVEMHDVKNRRTFLKRTKYEDLRLEDLFIGNKVNVFSRQLVLIDYGDQYTARQLGSRKEKTLALIKPDAVSKAGEIIEMINKSGFTITKLRMMTLTRKEAADFHVDHHSRPFYNELIQFITSGPVIAMEILRDDAICEWKRLLGPANSGLSRTDAPGSIRALFGTDGVRNAAHGPDTFASAAREMELFFPSSGGCGPANTAKFTNCTCCIIKPHAISEDLFIHYM

SEQ ID NO: 115 - DNA, 483 bp, Artificial Sequence
  NM23 P96S (cloned between NdeI and XhoI)
atggccaactgtgagcgtaccttcattgcgatcaaaccagatggggtccagcggggtcttgtgggagagattatcaagcgttttgagcagaaaggattccgccttgttggtctgaaattcatgcaagcttccgaagatcttctcaaggaacactacgttgacctgaaggaccgtccattctttgccggcctggtgaaatacatgcactcagggccggtagttgccatggtctgggaggggctgaatgtggtgaagacgggccgagtcatgctcggggagaccaactctgcagactccaagcctgggaccatccgtggagacttctgcatacaagttggcaggaacattatacatggcagtgattctgtggagagtgcagagaaggagatcggcttgtggtttcaccctgaggaactggtagattacacgagctgtgctcagaactggatctatgaactcgagcaccaccaccaccaccactga

SEQ ID NO: 116 - protein, 160 aa, Artificial Sequence
  NM23 P96S (cloned between NdeI and XhoI) with histidine tag at the C-terminus
MANCERTFIAIKPDGVQRGLVGEIIKRFEQKGFRLVGLKFMQASEDLLKEHYVDLKDRPFFAGLVKYMHSGPVVAMVWEGLNVVKTGRVMLGETNSADSKPGTIRGDFCIQVGRNIIHGSDSVESAEKEIGLWFHPEELVDYTSCAQNWIYELEHHHHHH

SEQ ID NO: 117 - DNA, 483 bp, Artificial Sequence
  NM23 P96S/S120G cloned between NdeI and XhoI
atggccaactgtgagcgtaccttcattgcgatcaaaccagatggggtccagcggggtcttgtgggagagattatcaagcgttttgagcagaaaggattccgccttgttggtctgaaattcatgcaagcttccgaagatcttctcaaggaacactacgttgacctgaaggaccgtccattctttgccggcctggtgaaatacatgcactcagggccggtagttgccatggtctgggaggggctgaatgtggtgaagacgggccgagtcatgctcggggagaccaactctgcagactccaagcctgggaccatccgtggagacttctgcatacaagttggcaggaacattatacatggcggtgattctgtggagagtgcagagaaggagatcggcttgtggtttcaccctgaggaactggtagattacacgagctgtgctcagaactggatctatgaactcgagcaccaccaccaccaccactga

SEQ ID NO: 118 - protein, 160 aa, Artificial Sequence
  NM23 P96S/S120G cloned between NdeI and XhoI with histidine tag at the C-terminus
MANCERTFIAIKPDGVQRGLVGEIIKRFEQKGFRLVGLKFMQASEDLLKEHYVDLKDRPFFAGLVKYMHSGPVVAMVWEGLNVVKTGRVMLGETNSADSKPGTIRGDFCIQVGRNIIHGGDSVESAEKEIGLWFHPEELVDYTSCAQNWIYELEHHHHHH

SEQ ID NO: 119 - DNA, 480 bp, Artificial Sequence
  NM23 P96S Delta C1 cloned between NdeI and XhoI
atggccaactgtgagcgtaccttcattgcgatcaaaccagatggggtccagcggggtcttgtgggagagattatcaagcgttttgagcagaaaggattccgccttgttggtctgaaattcatgcaagcttccgaagatcttctcaaggaacactacgttgacctgaaggaccgtccattctttgccggcctggtgaaatacatgcactcagggccggtagttgccatggtctgggaggggctgaatgtggtgaagacgggccgagtcatgctcggggagaccaactctgcagactccaagcctgggaccatccgtggagacttctgcatacaagttggcaggaacattatacatggcagtgattctgtggagagtgcagagaaggagatcggcttgtggtttcaccctgaggaactggtagattacacgagctgtgctcagaactggatctatctcgagcaccaccaccaccaccactga

SEQ ID NO: 120 - protein, 159 aa, Artificial Sequence
  NM23 P96S Delta C1 cloned between NdeI and XhoI with histidine tag at the C-terminus
MANCERTFIAIKPDGVQRGLVGEIIKRFEQKGFRLVGLKFMQASEDLLKEHYVDLKDRPFFAGLVKYMHSGPVVAMVWEGLNVVKTGRVMLGETNSADSKPGTIRGDFCIQVGRNIIHGSDSVESAEKEIGLWFHPEELVDYTSCAQNWIYLEHHHHHH

SEQ ID NO: 121 - DNA, 477 bp, Artificial Sequence
  NM23 P96S Delta C2 cloned between NdeI and XhoI
atggccaactgtgagcgtaccttcattgcgatcaaaccagatggggtccagcggggtcttgtgggagagattatcaagcgttttgagcagaaaggattccgccttgttggtctgaaattcatgcaagcttccgaagatcttctcaaggaacactacgttgacctgaaggaccgtccattctttgccggcctggtgaaatacatgcactcagggccggtagttgccatggtctgggaggggctgaatgtggtgaagacgggccgagtcatgctcggggagaccaactctgcagactccaagcctgggaccatccgtggagacttctgcatacaagttggcaggaacattatacatggcagtgattctgtggagagtgcagagaaggagatcggcttgtggtttcaccctgaggaactggtagattacacgagctgtgctcagaactggatcctcgagcaccaccaccaccaccactga

SEQ ID NO: 122 - protein, 158 aa, Artificial Sequence
  NM23 P96S Delta C2 cloned between NdeI and XhoI with histidine tag at the C-terminus
MANCERTFIAIKPDGVQRGLVGEIIKRFEQKGFRLVGLKFMQASEDLLKEHYVDLKDRPFFAGLVKYMHSGPVVAMVWEGLNVVKTGRVMLGETNSADSKPGTIRGDFCIQVGRNIIHGSDSVESAEKEIGLWFHPEELVDYTSCAQNWILEHHHHHH

SEQ ID NO: 123 - DNA, 465 bp, Artificial Sequence
  NM23 P96S Delta C6 cloned between NdeI and XhoI
atggccaactgtgagcgtaccttcattgcgatcaaaccagatggggtccagcggggtcttgtgggagagattatcaagcgttttgagcagaaaggattccgccttgttggtctgaaattcatgcaagcttccgaagatcttctcaaggaacactacgttgacctgaaggaccgtccattctttgccggcctggtgaaatacatgcactcagggccggtagttgccatggtctgggaggggctgaatgtggtgaagacgggccgagtcatgctcggggagaccaactctgcagactccaagcctgggaccatccgtggagacttctgcatacaagttggcaggaacattatacatggcagtgattctgtggagagtgcagagaaggagatcggcttgtggtttcaccctgaggaactggtagattacacgagctgtgctctcgagcaccaccaccaccaccactga

SEQ ID NO: 124 - protein, 154 aa, Artificial Sequence
  NM23 P96S Delta C6 cloned between NdeI and XhoI with histidine tag at the C-terminus
MANCERTFIAIKPDGVQRGLVGEIIKRFEQKGFRLVGLKFMQASEDLLKEHYVDLKDRPFFAGLVKYMHSGPVVAMVWEGLNVVKTGRVMLGETNSADSKPGTIRGDFCIQVGRNIIHGSDSVESAEKEIGLWFHPEELVDYTSCALEHHHHHH

SEQ ID NO: 125 - DNA, 480 bp, Artificial Sequence
  NM23 P96S Delta C1 /S120G cloned between NdeI and XhoI
atggccaactgtgagcgtaccttcattgcgatcaaaccagatggggtccagcggggtcttgtgggagagattatcaagcgttttgagcagaaaggattccgccttgttggtctgaaattcatgcaagcttccgaagatcttctcaaggaacactacgttgacctgaaggaccgtccattctttgccggcctggtgaaatacatgcactcagggccggtagttgccatggtctgggaggggctgaatgtggtgaagacgggccgagtcatgctcggggagaccaactctgcagactccaagcctgggaccatccgtggagacttctgcatacaagttggcaggaacattatacatggcggtgattctgtggagagtgcagagaaggagatcggcttgtggtttcaccctgaggaactggtagattacacgagctgtgctcagaactggatctatctcgagcaccaccaccaccaccactga

SEQ ID NO: 126 - protein, 159 aa, Artificial Sequence
  NM23 P96S Delta C1 /S120G cloned between NdeI and XhoI with histidine tag at the C-terminus
MANCERTFIAIKPDGVQRGLVGEIIKRFEQKGFRLVGLKFMQASEDLLKEHYVDLKDRPFFAGLVKYMHSGPVVAMVWEGLNVVKTGRVMLGETNSADSKPGTIRGDFCIQVGRNIIHGGDSVESAEKEIGLWFHPEELVDYTSCAQNWIYLEHHHHHH

SEQ ID NO: 127 - DNA, 477 bp, Artificial Sequence
  NM23 P96S Delta C2 /S120G cloned between NdeI and XhoI
atggccaactgtgagcgtaccttcattgcgatcaaaccagatggggtccagcggggtcttgtgggagagattatcaagcgttttgagcagaaaggattccgccttgttggtctgaaattcatgcaagcttccgaagatcttctcaaggaacactacgttgacctgaaggaccgtccattctttgccggcctggtgaaatacatgcactcagggccggtagttgccatggtctgggaggggctgaatgtggtgaagacgggccgagtcatgctcggggagaccaactctgcagactccaagcctgggaccatccgtggagacttctgcatacaagttggcaggaacattatacatggcggtgattctgtggagagtgcagagaaggagatcggcttgtggtttcaccctgaggaactggtagattacacgagctgtgctcagaactggatcctcgagcaccaccaccaccaccactga

SEQ ID NO: 128 - protein, 158 aa, Artificial Sequence
  NM23 P96S Delta C2 /S120G cloned between NdeI and XhoI with histidine tag at the C-terminus
MANCERTFIAIKPDGVQRGLVGEIIKRFEQKGFRLVGLKFMQASEDLLKEHYVDLKDRPFFAGLVKYMHSGPVVAMVWEGLNVVKTGRVMLGETNSADSKPGTIRGDFCIQVGRNIIHGGDSVESAEKEIGLWFHPEELVDYTSCAQNWILEHHHHHH

SEQ ID NO: 129 - DNA, 465 bp, Artificial Sequence
  NM23 P96S Delta C6 /S120G cloned between NdeI and XhoI
atggccaactgtgagcgtaccttcattgcgatcaaaccagatggggtccagcggggtcttgtgggagagattatcaagcgttttgagcagaaaggattccgccttgttggtctgaaattcatgcaagcttccgaagatcttctcaaggaacactacgttgacctgaaggaccgtccattctttgccggcctggtgaaatacatgcactcagggccggtagttgccatggtctgggaggggctgaatgtggtgaagacgggccgagtcatgctcggggagaccaactctgcagactccaagcctgggaccatccgtggagacttctgcatacaagttggcaggaacattatacatggcggtgattctgtggagagtgcagagaaggagatcggcttgtggtttcaccctgaggaactggtagattacacgagctgtgctctcgagcaccaccaccaccaccactga

SEQ ID NO: 130 - protein, 154 aa, Artificial Sequence
  NM23 P96S Delta C6 /S120G cloned between NdeI and XhoI with histidine tag at the C-terminus
MANCERTFIAIKPDGVQRGLVGEIIKRFEQKGFRLVGLKFMQASEDLLKEHYVDLKDRPFFAGLVKYMHSGPVVAMVWEGLNVVKTGRVMLGETNSADSKPGTIRGDFCIQVGRNIIHGGDSVESAEKEIGLWFHPEELVDYTSCALEHHHHHH

SEQ ID NO: 131 - DNA, 12 bp, Artificial Sequence
  Linkers
ggtggttctggt

SEQ ID NO: 132 - protein, 4 aa, Artificial Sequence
  Linkers
GGSG

SEQ ID NO: 133 - DNA, 22 bp, Artificial Sequence
  Linkers
  misc_feature (19)..(19): n is a, c, g, or t
gctgaagctgctgctaaangct

SEQ ID NO: 134 - protein, 8 aa, Artificial Sequence
  Linkers
AEAAAKNA

SEQ ID NO: 135 - DNA, 54 bp, Artificial Sequence
  Linkers
ggtgctggtggtgctggtggtgctggtgctggtggtgctggtgctggtgctggt

SEQ ID NO: 136 - protein, 18 aa, Artificial Sequence
  Linkers
GAGGAGGAGAGGAGAGAG

SEQ ID NO: 137 - DNA, 114 bp, Artificial Sequence
  Linkers
ggtgctggtggtgctggtggtgctggtgctggtggtgctggtgctggtgctggtgaacttggtgctggtggtgctggtggtgctggtgctggtggtgctggtgctggtgctggt

SEQ ID NO: 138 - protein, 38 aa, Artificial Sequence
  Linkers
GAGGAGGAGAGGAGAGAGELGAGGAGGAGAGGAGAGAG

SEQ ID NO: 139 - DNA, 24 bp, Artificial Sequence
  Linkers
ggtggtgctggtgctggtgctggt

SEQ ID NO: 140 - protein, 8 aa, Artificial Sequence
  Linkers
GGAGAGAG

SEQ ID NO: 141 - DNA, 39 bp, Artificial Sequence
  Linkers
ggttctggtggtggtggttctggtggtggtggttctggt

SEQ ID NO: 142 - protein, 13 aa, Artificial Sequence
  Linkers
GSGGGGSGGGGSG

SEQ ID NO: 143 - DNA, 12 bp, Artificial Sequence
  Linkers
cttgctgctgct

SEQ ID NO: 144 - protein, 4 aa, Artificial Sequence
  Linkers
LAAA

SEQ ID NO: 145 - DNA, 57 bp, Artificial Sequence
  Linkers
cttggtggtggtggttctggtggtggtggttctggtggtggtggttctgctgctgct

SEQ ID NO: 146 - protein, 19 aa, Artificial Sequence
  Linkers
LGGGGSGGGGSGGGGSAAA

SEQ ID NO: 147 - DNA, 75 bp, Artificial Sequence
  Linkers
ctttctggtggtggtggttctggtggtggtggttctggtggtggtggttctggtggtggtggttctgctgctgct

SEQ ID NO: 148 - protein, 25 aa, Artificial Sequence
  Linkers
LSGGGGSGGGGSGGGGSGGGGSAAA

SEQ ID NO: 149 - DNA, 31 bp, Artificial Sequence
  Linkers
  misc_feature (22)..(22): n is a, c, g, or t
cttgctgaagctgctgctaaangctgctgct

SEQ ID NO: 150 - protein, 11 aa, Artificial Sequence
  Linkers
LAEAAAKNAAA

SEQ ID NO: 151 - DNA, 120 bp, Artificial Sequence
  Linkers
ctttttaataaagaacaacaaaatgctttttatgaaattcttcatcttcctaatcttaatgaagaacaacgtaatggttttattcaatctcttaaagatgatccttctcaatctgctaat

SEQ ID NO: 152 - protein, 55 aa, Artificial Sequence
  Linkers
LFNKEQQNAFYEILHLPNLNEEQRNGFIQSLKDDPSQSANLLAEAKKLNDAQAAA

SEQ ID NO: 153 - DNA, 63 bp, Artificial Sequence
  Leader Sequence
aaatatcttcttcctactgctgctgctggtcttcttcttcttgctgctcaacctgctatggct

SEQ ID NO: 154 - protein, 21 aa, Artificial Sequence
  Leader Sequence
KYLLPTAAAGLLLLAAQPAMA

SEQ ID NO: 155 - DNA, 54 bp, Artificial Sequence
  Leader Sequence
atgaaatgggttacttttatttctcttctttttcttttttcttctgcttattct

SEQ ID NO: 156 - protein, 18 aa, Artificial Sequence
  Leader Sequence
MKWVTFISLLFLFSSAYS

SEQ ID NO: 157 - DNA, 66 bp, Artificial Sequence
  Leader Sequence
atggattttcaagttcaaattttttcttttcttcttatttctgcttctgttattatgtctcgtggt

SEQ ID NO: 158 - protein, 22 aa, Artificial Sequence
  Leader Sequence
MDFQVQIFSFLLISASVIMSRG